European Patent Application EP 4 650 438 A1, published November 19, 2025. Title: Cells having the phenotype of cardiac valve cells and the treatment of a valve defect. Applicant: Max-Planck-Gesellschaft zur Förderung der Wissenschaften e.V. The sequence listing filed with the application follows.

SEQUENCE LISTING (25 sequences)

SEQ ID NO: 1 - protein, 387 aa, Homo sapiens
  source 1..387: note = human EGR3 protein
MTGKLAEKLPVTMSSLLNQLPDNLYPEEIPSALNLFSGSSDSVVHYNQMATENVMDIGLTNEKPNPELSYSGSFQPAPGNKTVTYLGKFAFDSPSNWCQDNIISLMSAGILGVPPASGALSTQTSTASMVQPPQGDVEAMYPALPPYSNCGDLYSEPVSFHDPQGNPGLAYSPQDYQSAKPALDSNLFPMIPDYNLYHHPNDMGSIPEHKPFQGMDPIRVNPPPITPLETIKAFKDKQIHPGFGSLPQPPLTLKPIRPRKYPNRPSKTPLHERPHACPAEGCDRRFSRSDELTRHLRIHTGHKPFQCRICMRSFSRSDHLTTHIRTHTGEKPFACEFCGRKFARSDERKRHAKIHLKQKEKKAEKGGAPSASSAPPVSLAPVVTTCA

SEQ ID NO: 2 - RNA, 1164 nt, Homo sapiens
  source 1..1164: mol_type = mRNA; note = human EGR3 transcript
atgaccggcaaactcgccgagaagctgccggtgaccatgagcagtttgctaaaccaactgcctgacaatctgtaccccgaggagatccccagcgcgctcaacctcttctccggcagcagcgactcggtagtccattacaatcagatggctacagagaatgtaatggacatcggtctgaccaacgagaagcccaacccggaactctcttactccggctccttccagccagcccccggcaacaagaccgtgacctacttgggaaagttcgccttcgactccccttccaactggtgccaggacaacatcattagcctcatgagcgccggcatcttgggggtgcccccggcttcaggggcgctcagcacgcagacgtccacggccagcatggtgcagccaccgcagggtgacgtggaggccatgtatcccgcgctacccccctactccaactgcggcgacctctactcagagcccgtgtctttccacgacccccagggcaatcccgggctcgcctattccccccaggattaccaatcggccaagccggcgttggacagcaatctcttccccatgattcctgactacaacctctaccaccaccccaacgacatgggctccattccggagcacaagcccttccagggcatggaccccatccgggtcaacccgccccctattacccctctggagaccatcaaggcattcaaagacaagcagatccacccgggctttggcagcctgccccagccgccgctcaccctcaagcccatccggccccgcaagtaccccaaccggcctagcaagacaccgctccacgaacggccccacgcgtgcccggccgagggctgcgaccgccgtttcagccgttcggacgagctgacccggcacctgcgcatccacacgggccacaagcccttccagtgccggatctgcatgcggagcttcagccgcagcgaccacctcaccactcacatccgcactcatacgggcgagaagccctttgcctgcgagttctgcgggcgcaagtttgcgcgcagcgacgagcgcaagcgccacgccaagatccacctcaagcaaaaggagaagaaggcggagaagggcggtgcaccctctgcatcctcggcgccccccgtgtcgctggcccccgtggtcaccacctgcgcctga

SEQ ID NO: 3 - protein, 422 aa, Danio rerio
  source 1..422: note = Zebrafish Egr3 protein
MTGKLADKIPITMSSLINTIPDSLYPEEDIPTSMNIFANPDSISHYSQMNTDNIMDLGMGGEKGSGEIQYGSGSFQSGRSGQTVTYLGKFAFDTPPSGSIGGSGWCPDNNIISLVSAGILGVSPSPGNITTQTSSSSGSMGGQSSDMEQVYAPPLPAYSTCGEIYPEQVTFHHSPATSSSLPYPSSDYHTTSKPGMDGSLFSMIPDYNLFHHQGDVGVMEHKPFQTMDPIRVNPPPITPLETIRAFKDKQQIHPGFLGGQQHVSQHHQPSQTLALKPIRPRKYPNRPSKTPVHERPHACPAENCDRRFSRSDELTRHLRIHTGHKPFQCRICMRSFSRSDHLTTHIRTHTGEKPFSCEFCGRKFARSDERKRHAKVHLKQKDKKPTDKGSSAGAGGNHTSPPSSCGSAGPSSTNIMTVTTCA

SEQ ID NO: 4 - RNA, 1269 nt, Danio rerio
  source 1..1269: mol_type = mRNA; note = Zebrafish egr3 transcript
atgacaggtaaactagcggacaagatccctattaccatgagcagtttaatcaacaccatacctgacagtctctacccagaagaagacatcccaacttctatgaacattttcgcaaacccggactccatttcgcactactcgcagatgaatacagataatatcatggacttggggatgggcggcgagaagggcagcggagaaattcagtacggctccggcagcttccagtctgggcgaagtgggcagaccgtcacctacctgggcaagtttgcattcgacacccctccttcaggcagcatcggcggctccggctggtgtcccgacaacaacatcataagcctggtgagtgcaggcatcctaggggtgtccccttcacctggaaacatcaccacccagacgtcttcatccagcggcagcatgggtggccagtcttcagacatggagcaagtatacgcaccacccctacctgcctactccacctgtggagaaatatacccagagcaggtgacgttccaccacagtccggccacgtcctcatccttgccctacccgagctctgactaccacaccacctctaaaccaggcatggacggcagtctcttctccatgatcccagactacaacctcttccatcatcagggagacgtaggggtgatggagcataaaccctttcaaaccatggaccctatcagggtgaacccgcctcccataactcccctcgagaccattcgagcttttaaggataagcagcagattcatcccggcttcctcggtgggcaacagcacgtttcgcaacatcatcaaccctctcagacactagctctcaaacctatccgtccaagaaagtatcccaacaggccgagcaaaactccagtgcacgagagaccacatgcctgtccggccgagaactgtgaccggcgtttttcgcgatccgatgagttgacgcggcacctgcgcatccacacaggacacaaacccttccagtgccgcatctgcatgcggtccttcagtcgcagtgaccatctcaccacacacatccgcacacacaccggcgagaagccgttctcttgcgaattctgtggacgcaagtttgcgcggagcgacgagcgaaagcggcacgccaaggtgcacctcaaacagaaggacaagaaacccacggacaagggcagcagtgctggggcaggggggaaccacacttctcctcccagctcctgtgggagcgcaggacccagcagtactaacatcatgaccgtcaccacttgtgcatga

SEQ ID NO: 5 - RNA, 4514 nt, Homo sapiens
  source 1..4514: mol_type = mRNA; note = human EGR3 transcript
gggagcttttgggcagcagtgagcttgctaggaagcggcggggctggtggtggtggtagcagcggcggcagcggcggcagaggcggcggcggcggcggcggcggcggcggcggtggcggtggcggtggcggtggcagatcggggggcgggggggcggcgggcgcgtgtctgtttgtgagatcaatactgaggccgcgtccgacccccttgagccgagatccccccccagcccagcccccaccccaccccccgcacacgccccaccccccccacgacccagcctcataccgcaccagctgaggcacccaagaggattaccccctggggccctctcccgccccccaaaaaagagaagatcccctctcctggcccatcccttcccttcttccctcccccctccccccgaactttccctctcgcatgcttttcccctgcaccacggatcgcctctcggatgccgcttgcctggaagctgcgttaggagcgagcggcggcggtggcggcggtggcggcggcggcggcagctcgggagtgctatgaccggcaaactcgccgagaagctgccggtgaccatgagcagtttgctaaaccaactgcctgacaatctgtaccccgaggagatccccagcgcgctcaacctcttctccggcagcagcgactcggtagtccattacaatcagatggctacagagaatgtaatggacatcggtctgaccaacgagaagcccaacccggaactctcttactccggctccttccagccagcccccggcaacaagaccgtgacctacttgggaaagttcgccttcgactccccttccaactggtgccaggacaacatcattagcctcatgagcgccggcatcttgggggtgcccccggcttcaggggcgctcagcacgcagacgtccacggccagcatggtgcagccaccgcagggtgacgtggaggccatgtatcccgcgctacccccctactccaactgcggcgacctctactcagagcccgtgtctttccacgacccccagggcaatcccgggctcgcctattccccccaggattaccaatcggccaagccggcgttggacagcaatctcttccccatgattcctgactacaacctctaccaccaccccaacgacatgggctccattccggagcacaagcccttccagggcatggaccccatccgggtcaacccgccccctattacccctctggagaccatcaaggcattcaaagacaagcagatccacccgggctttggcagcctgccccagccgccgctcaccctcaagcccatccggccccgcaagtaccccaaccggcctagcaagacaccgctccacgaacggccccacgcgtgcccggccgagggctgcgaccgccgtttcagccgttcggacgagctgacccggcacctgcgcatccacacgggccacaagcccttccagtgccggatctgcatgcggagcttcagccgcagcgaccacctcaccactcacatccgcactcatacgggcgagaagccctttgcctgcgagttctgcgggcgcaagtttgcgcgcagcgacgagcgcaagcgccacgccaagatccacctcaagcaaaaggagaagaaggcggagaagggcggtgcaccctctgcatcctcggcgccccccgtgtcgctggcccccgtggtcaccacctgcgcctgaggatcgggcccccagatccccacttttcccctccagtgcctcccggctgctagcctgaaagcagcgggaaagccagccacggaggcgtaggggccgcgccctggcctctccatggacgtgcggccccttgcttccccttcgatgcccccggttcccaacctttcacgccggccagcggtcaggggccagggctggaggcgccttcccctcgcggtcccccacttagccaaggcgtgggggcggaaaggtggcgtctagcccgctttgttcagttcggatcgccttgatccaggggccgccgggccgcgccaaggacctgcaagggactgaaggcggagcccatccaaccctcgcccgacccaaacacctcattgtttcccccacgtctccctctataccccctcgaagactcgagagggggagggggtaaggagcgcaccaaagcgcagagcttgctgcccgccgcacgcacgcgcgcctgcgtgcggggatgcgcgcgagtgtgtgcgtgctcgcgtgtgtgtgtatgtgtgtgtgtgagtgtgtgtgtgtgcgcgcgcgcaagcgtgtgtgtttaagactcttgagctgaactgggctgtgtttaccccaaactcttccccacctcgggtccccaagccgctgggagatgtcccatgctgggggtccgcacgtggctggaggaggtggtcttccatccgctctgaaatcatgtttcttagagaaatgcctcggatgccgccgacgcggtgctgctgccgccgcttcgggtttggcccctcagaacccctccttttctgagcgcttccctcttaggcctcagggcagtttgatctgtggggagaaagagcagccatcgctgagcctgccttttaaaatatatgtgtatttccttagccccactctaagaaatctatgttcctgagtttgccccctgccctcccactccttccccttctcccctctaaaccttctcccatctctttcaaaatcttttcccagaaaggcaggcttcaaccagccactccagctttgtgtcttctctcaattacatagcaatttctccttcccaccatcatggggaagctggctctgcttttgccctttgtcatcaccaacacaacagatagaatttaaatataagtatatggtgtgcgtgtgtatgtatgtgtatgtatatgcatgcatgtgtataaagatgcacatgcgtacatatacataacatacacacaatatgtattcctagcaaaataaaatctctaaggtacttggttatccagtgcagtgcaccggaataaagagaatttgtaggcgtatacagctttaaatgatttattttttatgaaaatgttaactgatgagattatatctacatacgtgtgttatgtgtgtggatatagatgcacacatatctgtacatatacatgtgagtgtacatatatacacatatacacatctatgtatggatatgtgtgtatacacatatacacatctctgtccaaaatttcctcaaagatatggggattttttcatgaatccatgtggatgaatgaggtgtctcctttccatacccagtctcaccttctccccaccctacctcacctcttctcaggcacccctcttccccagctgtcctgccagcccttctcgtacagggtggctcctttgaagtggagtaatagggaaggttgctctctgccacagcttgcagcatggtcttgactgaatgtactgttcctgttagcgttacttctcctgtggtcagtaagttgcccagagagaaggaacaaaggtctggagtttacagaatgtctgtttttaaagtcactttatgcgttttccacttttttcttttttaagaaaaagaagtaccatttttgttttgttttgttttgatttttggtggtggataaataatactaaaaggactctagtggaaaggggggatatcgaagagcagggggttgtgaatttccaggtacttggactttttgtagaaggagagagaagaagatgaagtttgccaggagggcccatattttttcagctgaagggtaaaatctttctttgcagagacagtattttgctgaatactttttataatgtgatgattattaaaaaagcaaaaattttggtcacttccaagctagaaggaggaatcagataccctttaatattttttcctcgctccttctggtatatgcatgtcactgcatgataattgagttttcctttgttttaataaaactgttctcagacattaagctaaactaagagaaaaataactttgttgccaaaaggttgtgctatccagattttttatatgtctgcatgtttaaaaaaaaaaagcaacaaaagaaaatgcactctaacttatgtgaactgagagaaaaaaatcaggttttaaacaggaaaacctatggggaatgatattttttgaaagacttttgtataaagttgagtacttagaaaaaagacaaaccagatgtaatatattttgtggatgtttttatttcttggatttatagtaccttatactaaggttaaaaaaatatgcttgatattgtgaaaaggtgaaattcttcaccaacatttcatttgctcctttgtcatattgtaatgccaatataatatagttaatgaaaacagcatttttaaaaaccgaaatattgaaatggtgtaatgttgtaccatttgcactgtgagcaaatgctaatacagtaaatatattgtgtttgctgacaatcagccggcctataaatctccttattttatttcttgtttttatagcataaagctttagtttggcctgtt

SEQ ID NO: 6 - RNA, 3258 nt, Danio rerio
  source 1..3258: mol_type = mRNA; note = Zebrafish egr3 transcript
cacgcacaaaaaaacaaccctcctcgcgaagagacatcagcgccgtgcccgtcgcgcgctcggatttaatttccaaggcttcgagggtctcctgctgtcgcttttcgggtgatttctgaagacggatcgggattgaacacctgtgcgcgctcattaatgacagcctgaagaactgctatgacaggtaaactagcggacaagatccctattaccatgagcagtttaatcaacaccatacctgacagtctctacccagaagaagacatcccaacttctatgaacattttcgcaaacccggactccatttcgcactactcgcagatgaatacagataatatcatggacttggggatgggcggcgagaagggcagcggagaaattcagtacggctccggcagcttccagtctgggcgaagtgggcagaccgtcacctacctgggcaagtttgcattcgacacccctccttcaggcagcatcggcggctccggctggtgtcccgacaacaacatcataagcctggtgagtgcaggcatcctaggggtgtccccttcacctggaaacatcaccacccagacgtcttcatccagcggcagcatgggtggccagtcttcagacatggagcaagtatacgcaccacccctacctgcctactccacctgtggagaaatatacccagagcaggtgacgttccaccacagtccggccacgtcctcatccttgccctacccgagctctgactaccacaccacctctaaaccaggcatggacggcagtctcttctccatgatcccagactacaacctcttccatcatcagggagacgtaggggtgatggagcataaaccctttcaaaccatggaccctatcagggtgaacccgcctcccataactcccctcgagaccattcgagcttttaaggataagcagcagattcatcccggcttcctcggtgggcaacagcacgtttcgcaacatcatcaaccctctcagacactagctctcaaacctatccgtccaagaaagtatcccaacaggccgagcaaaactccagtgcacgagagaccacatgcctgtccggccgagaactgtgaccggcgtttttcgcgatccgatgagttgacgcggcacctgcgcatccacacaggacacaaacccttccagtgccgcatctgcatgcggtccttcagtcgcagtgaccatctcaccacacacatccgcacacacaccggcgagaagccgttctcttgcgaattctgtggacgcaagtttgcgcggagcgacgagcgaaagcggcacgccaaggtgcacctcaaacagaaggacaagaaacccacggacaagggcagcagtgctggggcaggggggaaccacacttctcctcccagctcctgtgggagcgcaggacccagcagtactaacatcatgaccgtcaccacttgtgcatgagatggacttgaaaagtaagactgtgaggtgaaaaaaaaccgaagttttctttctcctctttacatacacttgactctctccctctcactatattcatccggtttctattgattatggtggcgcatttctgtagccactactgtggtaggtcaagtgagtggggagtaagtggacttggatgggaagcagagggcgtcaaagatgacagttcaagcagtcgggtcagtccacagaaagagcacttacagatgcagcacagtcaactctcagctccggagaccagagcgtctcttcagagtttaggtctacttcttgtattttggttcgttggatgaaaaaaaaaaaagtgcactttcatttgcttaatgtttcgcagtcttttttaaaatgattgttaattatttaatgtttctgtgttattgttgttgtttttcaagagaatgtgccaaatgtatttaaatacagcagatgatttaaaaacgatatattgtttgtatttacctaataacttcggttcagacattaatttggggaaagcctatgagctctaaacgtgacgttaaaagtctgattatttacatattttgaaatccggatgacgtttattatcagcgacggactttcagtgcaataaggaaagaaaaacaacaacaaaaacaacaataaaacgcagtctggctcactttcacatgtttaccttctggggacttaatgaaggcacgtctttgcctttattaagcgcgcatataagggccaaacacaatacgattaaaagattttgcctttctgtttttgctgcatgcacctagtgtcatgtctagtactgagaagattgcatcagtcatgatcgacctacagcaatacgcatccaactcaaaccatgcagagtgtcatttaaaaaaattgacctatttttatgtgaaaactgtccctctgttgtccttatcgtcattgttttactgaacggttgcatttcctcatccaatattgttcatggggtccctttttacgcacattatatattcagcacgcatttgaacacacatgtacacacaaacgaaatcagccaaaattatggtaatgcttgcctgcgagcatcaccactgggcaggattgatcttaggagtcattgttttgcatttttaccggctgaggccctgcctgctatatgcatgccattcaagttgtttttggatgggaacagttccgacatttatactgctctcaggggcagcaccgtaatgtggtatctccacggttactcatatcccgatcatgcctagagattctgaatattaacgacgagaacgcgagggggttttgtacagataattttacaaacatattactacatgttttatacttggaatgtacaaagcgatgtctttcagtattacgatgtctgtctgtacacgtgtgtatgtgtgtgtgtgtgtgcgcgtgtataaatgtgtgcgtatgctaatgcacacacaaacacccgcatacttagattttacattgactgaatgttgaaacaaagggtgtgtttacatttttgttggctttttttctgttttcgagacgtgtacatagtgttgaatgtttttttgtaagtgtgtgtgtgtgtgtgtgagagagaaagaatgagtgtgtgagtgcaggaaaatctgagtactgacagtgtcaaatgtgatgcattctccggcatttcttcaaagtcttaaatattaactgttattagtgcgaattctgacttgcagacacactgaatgatgtgtttaataaatgaataaacagtaagattatttgctgaaaaaagcaaaacaaaaa

SEQ ID NO: 7 - DNA, 59 bp, synthetic construct
  source 1..59: mol_type = other DNA; note = Wild-type
ctgctccgccgtgcgcttatcttcctgcgcttgcctgcgagcatcaccactgggcagga

SEQ ID NO: 8 - DNA, 22 bp, synthetic construct
  source 1..22: mol_type = other DNA; note = egr3 bns522
ctgctccgccgactgggcagga

SEQ ID NO: 9 - DNA, 51 bp, synthetic construct
  source 1..51: mol_type = other DNA; note = Wild-type
ttccaccacagtccggccacgtcctcatccttgccctacccgagctctgac

SEQ ID NO: 10 - protein, 17 aa, synthetic construct
  source 1..17: note = Wild-type
FHHSPATSSSLPYPSSD

SEQ ID NO: 11 - DNA, 40 bp, synthetic construct
  source 1..40: mol_type = other DNA; note = egr3 bns577
ttccaccacgtcctcatccttgccctacccgagctctgac

SEQ ID NO: 12 - protein, 12 aa, synthetic construct
  source 1..12: note = egr3 bns577
FHHVLILALPEL

SEQ ID NO: 13 - protein, 101 aa, synthetic construct
  source 1..101: note = sp|P26632|EGR1_DANRE
LIKPSRMRKYPNRPSKTPPHERPYACPVETCDRRFSRSDELTRHIRIHTGQKPFQCRICMRNFSRSDHLTTHIRTHTGEKPFACEICGRKFARSDERKRHT

SEQ ID NO: 14 - protein, 101 aa, synthetic construct
  source 1..101: note = sp|P08046|EGR1_MOUSE
LIKPSRMRKYPNRPSKTPPHERPYACPVESCDRRFSRSDELTRHIRIHTGQKPFQCRICMRNFSRSDHLTTHIRTHTGEKPFACDICGRKFARSDERKRHT

SEQ ID NO: 15 - protein, 101 aa, synthetic construct; identical to SEQ ID NO: 14
  source 1..101: note = sp|P18146|EGR1_HUMAN

SEQ ID NO: 16 - protein, 102 aa, synthetic construct
  source 1..102: note = tr|Q6DG27|Q6DG27_DANRE
LALKPIRPRKYPNRPSKTPVHERPHACPAENCDRRFSRSDELTRHLRIHTGHKPFQCRICMRSFSRSDHLTTHIRTHTGEKPFSCEFCGRKFARSDERKRHA

SEQ ID NO: 17 - protein, 101 aa, synthetic construct
  source 1..101: note = sp|P43300|EGR3_MOUSE
TLKPIRPRKYPNRPSKTPLHERPHACPAEGCDRRFSRSDELTRHLRIHTGHKPFQCRICMRSFSRSDHLTTHIRTHTGEKPFACEFCGRKFARSDERKRHA

SEQ ID NO: 18 - protein, 101 aa, synthetic construct; identical to SEQ ID NO: 17
  source 1..101: note = sp|Q06889|EGR3_HUMAN

SEQ ID NO: 19 - protein, 102 aa, synthetic construct
  source 1..102: note = tr|E7F266|E7F266_DANRE
PLRPILRPRKYPNRPCKTPVHERPYPCPAEGCDRRFSRSDELTRHVRIHTGHKPFQCRICMRSFSRSDHLTTHIRTHTGEKPFSCDFCGRKFARSDERRRHT

SEQ ID NO: 20 - protein, 102 aa, synthetic construct
  source 1..102: note = sp|Q05159|EGR2B_DANRE
PLRPILRPRKYPNRPSKTPVHERPYPCPAEGCDRRFSRSDELTRHIRIHTGHKPFQCRICMRNFSRSDHLTTHIRTHTGEKPFACDFCGRKFARSDERKRHT

SEQ ID NO: 21 - protein, 102 aa, synthetic construct
  source 1..102: note = sp|P08152|EGR2_MOUSE
PLRPILRPRKYPNRPSKTPVHERPYPCPAEGCDRRFSRSDELTRHIRIHTGHKPFQCRICMRNFSRSDHLTTHIRTHTGEKPFACDYCGRKFARSDERKRHT

SEQ ID NO: 22 - protein, 102 aa, synthetic construct; identical to SEQ ID NO: 21
  source 1..102: note = sp|P11161|EGR2_HUMAN

SEQ ID NO: 23 - protein, 95 aa, synthetic construct
  source 1..95: note = tr|A9JTG0|A9JTG0_DANRE
AQRSKPRARKGAAREKPFSCPVESCERRFSRSDELNRHVRIHTGHKPFQCRVCLRCFSRSDHLTTHMRTHTGEKPFSCDVCARRFARSDERKRHM

SEQ ID NO: 24 - protein, 102 aa, synthetic construct
  source 1..102: note = sp|Q9WUF2|EGR4_MOUSE
ARRKGRRGGKCSARCFCPRPHVKAFACPVESCVRSFARSDELNRHLRIHTGHKPFQCRICLRNFSRSDHLTTHVRTHTGEKPFACDVCGRRFARSDEKKRHS

SEQ ID NO: 25 - protein, 102 aa, synthetic construct
  source 1..102: note = sp|Q05215|EGR4_HUMAN
ARRKGRRGGKCSTRCFCPRPHAKAFACPVESCVRSFARSDELNRHLRIHTGHKPFQCRICLRNFSRSDHLTTHVRTHTGEKPFACDVCGRRFARSDEKKRHS